European Patent Specification EP 3 558 368 B1, published November 12, 2025. Title: ADAM9-Binding Molecules, and Methods of Use Thereof. Applicant: MacroGenics, Inc. Loo, Deryk Scribner, Juniper Barat, Bhaswati Diedrich, Gundo Johnson, Leslie Bonvini, Ezio. The sequence listing filed with the application follows.

SEQUENCE LISTING (207 sequences)

SEQ ID NO: 1 - protein, 217 aa, Homo sapiens
  MISC_FEATURE (1)..(200): CH2-CH3 Domain of Human IgG1
  MISC_FEATURE (200)..(200): Xaa is Lysine (K) or is Absent
  misc_feature (217)..(217): Xaa can be any naturally occurring amino acid
APELLGGPSVFLFPPKPKDTLMISRTPEVTCVVVDVSHEDPEVKFNWYVDGVEVHNAKTKPREEQYNSTYRVVSVLTVLHQDWLNGKEYKCKVSNKALPAPIEKTISKAKGQPREPQVYTLPPSREEMTKNQVSLTCLVKGFYPSDIAVEWESNGQPENNYKTTPPVLDSDGSFFLYSKLTVDKSRWQQGNVFSCSVMHEALHNHYTQKSLSLSPGX

SEQ ID NO: 2 - protein, 216 aa, Homo sapiens
  MISC_FEATURE (1)..(216): CH2-CH3 Domain of Human IgG2
  MISC_FEATURE (216)..(216): Xaa is Lysine (K) or is Absent
APPVAGPSVFLFPPKPKDTLMISRTPEVTCVVVDVSHEDPEVQFNWYVDGVEVHNAKTKPREEQFNSTFRVVSVLTVVHQDWLNGKEYKCKVSNKGLPAPIEKTISKTKGQPREPQVYTLPPSREEMTKNQVSLTCLVKGFYPSDISVEWESNGQPENNYKTTPPMLDSDGSFFLYSKLTVDKSRWQQGNVFSCSVMHEALHNHYTQKSLSLSPGX

SEQ ID NO: 3 - protein, 217 aa, Homo sapiens
  MISC_FEATURE (1)..(217): CH2-CH3 Domain of Human IgG3
  MISC_FEATURE (217)..(217): Xaa is Lysine (K) or is Absent
APELLGGPSVFLFPPKPKDTLMISRTPEVTCVVVDVSHEDPEVQFKWYVDGVEVHNAKTKPREEQYNSTFRVVSVLTVLHQDWLNGKEYKCKVSNKALPAPIEKTISKTKGQPREPQVYTLPPSREEMTKNQVSLTCLVKGFYPSDIAVEWESSGQPENNYNTTPPMLDSDGSFFLYSKLTVDKSRWQQGNIFSCSVMHEALHNRFTQKSLSLSPGX

SEQ ID NO: 4 - protein, 217 aa, Homo sapiens
  MISC_FEATURE (1)..(217): CH2-CH3 Domain of Human IgG4
  MISC_FEATURE (217)..(217): Xaa is Lysine (K) or is Absent
APEFLGGPSVFLFPPKPKDTLMISRTPEVTCVVVDVSQEDPEVQFNWYVDGVEVHNAKTKPREEQFNSTYRVVSVLTVLHQDWLNGKEYKCKVSNKGLPSSIEKTISKAKGQPREPQVYTLPPSQEEMTKNQVSLTCLVKGFYPSDIAVEWESNGQPENNYKTTPPVLDSDGSFFLYSRLTVDKSRWQEGNVFSCSVMHEALHNHYTQKSLSLSLGX

SEQ ID NO: 5 - protein, 819 aa, Homo sapiens
  MISC_FEATURE (1)..(819): Representative Human ADAM9 Polypeptide (NCBI Sequence NP_003807)
  SIGNAL (1)..(28): Signal Sequence
MGSGARFPSGTLRVRWLLLLGLVGPVLGAARPGFQQTSHLSSYEIITPWRLTRERREAPRPYSKQVSYVIQAEGKEHIIHLERNKDLLPEDFVVYTYNKEGTLITDHPNIQNHCHYRGYVEGVHNSSIALSDCFGLRGLLHLENASYGIEPLQNSSHFEHIIYRMDDVYKEPLKCGVSNKDIEKETAKDEEEEPPSMTQLLRRRRAVLPQTRYVELFIVVDKERYDMMGRNQTAVREEMILLANYLDSMYIMLNIRIVLVGLEIWTNGNLINIVGGAGDVLGNFVQWREKFLITRRRHDSAQLVLKKGFGGTAGMAFVGTVCSRSHAGGINVFGQITVETFASIVAHELGHNLGMNHDDGRDCSCGAKSCIMNSGASGSRNFSSCSAEDFEKLTLNKGGNCLLNIPKPDEAYSAPSCGNKLVDAGEECDCGTPKECELDPCCEGSTCKLKSFAECAYGDCCKDCRFLPGGTLCRGKTSECDVPEYCNGSSQFCQPDVFIQNGYPCQNNKAYCYNGMCQYYDAQCQVIFGSKAKAAPKDCFIEVNSKGDRFGNCGFSGNEYKKCATGNALCGKLQCENVQEIPVFGIVPAIIQTPSRGTKCWGVDFQLGSDVPDPGMVNEGTKCGAGKICRNFQCVDASVLNYDCDVQKKCHGHGVCNSNKNCHCENGWAPPNCETKGYGGSVDSGPTYNEMNTALRDGLLVFFFLIVPLIVCAIFIFIKRDQLWRSYFRKKRSQTYESDGKNQANPSRQPGSVPRHVSPVTPPREVPIYANRFAVPTYAAKQPQQFPSRPPPPQPKVSSQGNLIPARPAPAPPLYSSLT

SEQ ID NO: 6 - protein, 819 aa, Macaca fascicularis
  MISC_FEATURE (1)..(819): Representative Cynomolgus Monkey ADAM9 Polypeptide (NCBI Sequence XM_005563126.2)
  SIGNAL (1)..(28): Possible Signal Sequence
MGSGVGSPSGTLRVRWLLLLCLVGPVLGAARPGFQQTSHLSSYEIITPWRLTRERREAPRPYSKQVSYLIQAEGKEHIIHLERNKDLLPEDFVVYTYNKEGTVITDHPNIQNHCHFRGYVEGVYNSSVALSNCFGLRGLLHLENASYGIEPLQNSSHFEHIIYRMDDVHKEPLKCGVSNKDIEKETTKDEEEEPPSMTQLLRRRRAVLPQTRYVELFIVVDKERYDMMGRNQTAVREEMILLANYLDSMYIMLNIRIVLVGLEIWTNGNLINIAGGAGDVLGNFVQWREKFLITRRRHDSAQLVLKKGFGGTAGMAFVGTVCSRSHAGGINVFGHITVETFASIVAHELGHNLGMNHDDGRDCSCGAKSCIMNSGASGSRNFSSCSAEDFEKLTLNKGGNCLLNIPKPDEAYSAPSCGNKLVDAGEECDCGTPKECELDPCCEGSTCKLKSFAECAYGDCCKDCRFLPGGTLCRGKTSECDVPEYCNGSSQFCQPDVFIQNGYPCQNNKAYCYNGMCQYYDAQCQVIFGSKAKAAPKDCFIEVNSKGDRFGNCGFSGNEYKKCATGNALCGKLQCENVQEIPVFGIVPAIIQTPSRGTKCWGVDFQLGSDVPDPGMVNEGTKCGADKICRNFQCVDASVLNYDCDIQKKCHGHGVCNSNKNCHCENGWAPPNCETKGYGGSVDSGPTYNEMNTALRDGLLVFFFLIVPLIVCAIFIFIKRDQLWRRYFRKKRSQTYESDGKNQANPSRQPVSVPRHVSPVTPPREVPIYANRFPVPTYAAKQPQQFPSRPPPPQPKVSSQGNLIPARPAPAPPLYSSLT

SEQ ID NO: 7 - protein, 123 aa, Mus musculus
  MISC_FEATURE (1)..(123): VH Domain of Murine Anti-ADAM9 Antibody MAB-A
QVQLQQPGAELVKPGASVKLSCKASGYTFTSYWMHWVKQRPGQGLEWIGEIIPINGHTNYNEKFKSKATLTLDKSSSTAYMQLSSLASEDSAVYYCARGGYYYYGSRDYFDYWGQGTTLTVSS

SEQ ID NO: 8 - protein, 5 aa, Mus musculus
  MISC_FEATURE (1)..(5): CDRH1 Domain of Anti-ADAM9 Antibody MAB-A
SYWMH

SEQ ID NO: 9 - protein, 17 aa, Mus musculus
  MISC_FEATURE (1)..(17): CDRH2 Domain of Anti-ADAM9 Antibody MAB-A
EIIPINGHTNYNEKFKS

SEQ ID NO: 10 - protein, 14 aa, Mus musculus
  MISC_FEATURE (1)..(14): CDRH3 Domain of Anti-ADAM9 Antibody MAB-A
GGYYYYGSRDYFDY

SEQ ID NO: 11 - protein, 111 aa, Mus musculus
  MISC_FEATURE (1)..(111): VL Domain of Murine Anti-ADAM9 Antibody MAB-A
DIVLTQSPASLAVSLGQRATISCKASQSVDYDGDSYMNWYQQIPGQPPKLLIYAASDLESGIPARFSGSGSGTDFTLNIHPVEEEDAATYYCQQSHEDPFTFGGGTKLEIK

SEQ ID NO: 12 - protein, 15 aa, Mus musculus
  MISC_FEATURE (1)..(15): CDRL1 Domain of Anti-ADAM9 Antibody MAB-A
KASQSVDYDGDSYMN

SEQ ID NO: 13 - protein, 7 aa, Mus musculus
  MISC_FEATURE (1)..(7): CDRL2 Domain of Anti-ADAM9 Antibody MAB-A
AASDLES

SEQ ID NO: 14 - protein, 9 aa, Mus musculus
  MISC_FEATURE (1)..(9): CDRL3 Domain of Anti-ADAM9 Antibody MAB-A
QQSHEDPFT

SEQ ID NO: 15 - protein, 123 aa, Artificial Sequence
  Humanized/Optimized VH Domain of Murine Anti-ADAM9 Antibody MAB-A
  MISC_FEATURE (34)..(34): XAA is Methionine (M) or Isoleucine (I)
  MISC_FEATURE (55)..(55): XAA is Asparagine (N) or Phenylalanine (F)
  MISC_FEATURE (63)..(63): XAA is Lysine (K) or Arginine (R)
  MISC_FEATURE (65)..(65): XAA is Lysine (K) or Glutamine (Q)
  MISC_FEATURE (66)..(66): XAA is Serine (S) or Glycine (E)
  MISC_FEATURE (105)..(105): XAA is Proline (P), Phenylalanine (F), Tyrosine (Y), Tryptophan (W), Isoleuciine (I), Leucine (L), Valine (V), Threonine (T), Glycine (G) or Aspartate (D)
  MISC_FEATURE (106)..(106): XAA is Lysine (K), Arginine (R), Glycine (G), Asparagine (N), Histidine (H), or Serine (S)
  MISC_FEATURE (107)..(107): XAA is Phenylalanine (F), Methionine (M), Serine (S), Lysine (K) or Asparagine (N)
  MISC_FEATURE (108)..(108): XAA is Glycine (G) or Alanine (A)
  MISC_FEATURE (109)..(109): XAA is Valine (V), Threonine (T), Tryptophan (W) or Phenylalanine (F)
  MISC_FEATURE (109)..(109): XAA is Methionine (M), Leucine (L) or Lysine (K)
  misc_feature (110)..(110): Xaa can be any naturally occurring amino acid
EVQLVESGGGLVKPGGSLRLSCAASGFTFSSYWXHWVRQAPGKGLEWVGEIIPIXGHTNYNEXFXXRFTISLDNSKNTLYLQMGSLRAEDTAVYYCARGGYYYYXXXXXXDYWGQGTTVTVSS

SEQ ID NO: 16 - protein, 123 aa, Artificial Sequence
  VH(1) Domain of Humanized/Optimized Anti-ADAM9 Antibody hMAB-A (hMAB-A VH(1))
EVQLVESGGGLVKPGGSLRLSCAASGFTFSSYWMHWVRQAPGKGLEWVGEIIPINGHTNYNEKFKSRFTISLDNSKNTLYLQMGSLRAEDTAVYYCARGGYYYYGSRDYFDYWGQGTTVTVSS

SEQ ID NO: 17 - protein, 123 aa, Artificial Sequence
  VH(2) Domain of Humanized/Optimized Anti-ADAM9 Antibody hMAB-A (hMAB-A VH(2))
EVQLVESGGGLVKPGGSLRLSCAASGFTFSSYWMHWVRQAPGKGLEWVGEIIPIFGHTNYNEKFKSRFTISLDNSKNTLYLQMGSLRAEDTAVYYCARGGYYYYGSRDYFDYWGQGTTVTVSS

SEQ ID NO: 18 - protein, 123 aa, Artificial Sequence
  VH(3) Domain of Humanized/Optimized Anti-ADAM9 Antibody hMAB-A (hMAB-A VH(3))
EVQLVESGGGLVKPGGSLRLSCAASGFTFSSYWMHWVRQAPGKGLEWVGEIIPIFGHTNYNERFQGRFTISLDNSKNTLYLQMGSLRAEDTAVYYCARGGYYYYGSRDYFDYWGQGTTVTVSS

SEQ ID NO: 19 - protein, 123 aa, Artificial Sequence
  VH(4) Domain of Humanized/Optimized Anti-ADAM9 Antibody hMAB-A (hMAB-A VH(4))
EVQLVESGGGLVKPGGSLRLSCAASGFTFSSYWIHWVRQAPGKGLEWVGEIIPIFGHTNYNERFQGRFTISLDNSKNTLYLQMGSLRAEDTAVYYCARGGYYYYGSRDYFDYWGQGTTVTVSS

SEQ ID NO: 20 - protein, 123 aa, Artificial Sequence
  VH(2A) Domain of Humanized/Optimized Anti-ADAM9 Antibody hMAB-A (hMAB-A VH(2A))
EVQLVESGGGLVKPGGSLRLSCAASGFTFSSYWMHWVRQAPGKGLEWVGEIIPIFGHTNYNEKFKSRFTISLDNSKNTLYLQMGSLRAEDTAVYYCARGGYYYYFNSGTLDYWGQGTTVTVSS

SEQ ID NO: 21 - protein, 123 aa, Artificial Sequence
  VH(2B) Domain of Humanized/Optimized Anti-ADAM9 Antibody hMAB-A (hMAB-A VH(2B))
EVQLVESGGGLVKPGGSLRLSCAASGFTFSSYWMHWVRQAPGKGLEWVGEIIPIFGHTNYNEKFKSRFTISLDNSKNTLYLQMGSLRAEDTAVYYCARGGYYYYIGKGVLDYWGQGTTVTVSS

SEQ ID NO: 22 - protein, 123 aa, Artificial Sequence
  VH(2C) Domain of Humanized/Optimized Anti-ADAM9 Antibody hMAB-A (hMAB-A VH(2C))
EVQLVESGGGLVKPGGSLRLSCAASGFTFSSYWMHWVRQAPGKGLEWVGEIIPIFGHTNYNEKFKSRFTISLDNSKNTLYLQMGSLRAEDTAVYYCARGGYYYYPRFGWLDYWGQGTTVTVSS

SEQ ID NO: 23 - protein, 123 aa, Artificial Sequence
  VH(2D) Domain of Humanized/Optimized Anti-ADAM9 Antibody hMAB-A (hMAB-A VH(2D))
EVQLVESGGGLVKPGGSLRLSCAASGFTFSSYWMHWVRQAPGKGLEWVGEIIPIFGHTNYNEKFKSRFTISLDNSKNTLYLQMGSLRAEDTAVYYCARGGYYYYTGKGVLDYWGQGTTVTVSS

SEQ ID NO: 24 - protein, 123 aa, Artificial Sequence
  VH(2E) Domain of Humanized/Optimized Anti-ADAM9 Antibody hMAB-A (hMAB-A VH(2E))
EVQLVESGGGLVKPGGSLRLSCAASGFTFSSYWMHWVRQAPGKGLEWVGEIIPIFGHTNYNEKFKSRFTISLDNSKNTLYLQMGSLRAEDTAVYYCARGGYYYYDSNAVLDYWGQGTTVTVSS

SEQ ID NO: 25 - protein, 123 aa, Artificial Sequence
  VH(2F) Domain of Humanized/Optimized Anti-ADAM9 Antibody hMAB-A (hMAB-A VH(2F))
EVQLVESGGGLVKPGGSLRLSCAASGFTFSSYWMHWVRQAPGKGLEWVGEIIPIFGHTNYNEKFKSRFTISLDNSKNTLYLQMGSLRAEDTAVYYCARGGYYYYFHSGTLDYWGQGTTVTVSS

SEQ ID NO: 26 - protein, 123 aa, Artificial Sequence
  VH(2G) Domain of Humanized/Optimized Anti-ADAM9 Antibody hMAB-A (hMAB-A VH(2G))
EVQLVESGGGLVKPGGSLRLSCAASGFTFSSYWMHWVRQAPGKGLEWVGEIIPIFGHTNYNEKFKSRFTISLDNSKNTLYLQMGSLRAEDTAVYYCARGGYYYYFNKAVLDYWGQGTTVTVSS

SEQ ID NO: 27 - protein, 123 aa, Artificial Sequence
  VH(2H) Domain of Humanized/Optimized Anti-ADAM9 Antibody hMAB-A (hMAB-A VH(2H))
EVQLVESGGGLVKPGGSLRLSCAASGFTFSSYWMHWVRQAPGKGLEWVGEIIPIFGHTNYNEKFKSRFTISLDNSKNTLYLQMGSLRAEDTAVYYCARGGYYYYGGSGVLDYWGQGTTVTVSS

SEQ ID NO: 28 - protein, 123 aa, Artificial Sequence
  VH(2I) Domain of Humanized/Optimized Anti-ADAM9 Antibody hMAB-A (hMAB-A VH(2I))
EVQLVESGGGLVKPGGSLRLSCAASGFTFSSYWMHWVRQAPGKGLEWVGEIIPIFGHTNYNEKFKSRFTISLDNSKNTLYLQMGSLRAEDTAVYYCARGGYYYYPRQGFLDYWGQGTTVTVSS

SEQ ID NO: 29 - protein, 123 aa, Artificial Sequence
  VH(2J) Domain of Humanized/Optimized Anti-ADAM9 Antibody hMAB-A (hMAB-A VH(2J))
EVQLVESGGGLVKPGGSLRLSCAASGFTFSSYWMHWVRQAPGKGLEWVGEIIPIFGHTNYNEKFKSRFTISLDNSKNTLYLQMGSLRAEDTAVYYCARGGYYYYYNSGTLDYWGQGTTVTVSS

SEQ ID NO: 30 - protein, 30 aa, Artificial Sequence
  FRH1 Domain of Humanized/Optimized Murine Anti-ADAM9 Antibody MAB-A
EVQLVESGGGLVKPGGSLRLSCAASGFTFS

SEQ ID NO: 31 - protein, 14 aa, Artificial Sequence
  FRH2 Domain of Humanized/Optimized Murine Anti-ADAM9 Antibody MAB-A
WVRQAPGKGLEWVG

SEQ ID NO: 32 - protein, 32 aa, Artificial Sequence
  FRH3 Domain of Humanized/Optimized Murine Anti-ADAM9 Antibody MAB-A
RFTISLDNSKNTLYLQMGSLRAEDTAVYYCAR

SEQ ID NO: 33 - protein, 11 aa, Artificial Sequence
  FRH4 Domain of Humanized/Optimized Murine Anti-ADAM9 Antibody MAB-A
WGQGTTVTVSS

SEQ ID NO: 34 - protein, 5 aa, Artificial Sequence
  Alternative CDRH1 Domain of Anti-ADAM9-Antibody MAB-A
SYWIH

SEQ ID NO: 35 - protein, 17 aa, Artificial Sequence
  Alternative CDRH2 Domain of Anti-ADAM9-Antibody MAB-A
EIIPIFGHTNYNEKFKS

SEQ ID NO: 36 - protein, 17 aa, Artificial Sequence
  Alternative CDRH2 Domain of Anti-ADAM9-Antibody MAB-A
EIIPIFGHTNYNERFQG

SEQ ID NO: 37 - protein, 14 aa, Artificial Sequence
  Alternative CDRH3 Domain of Anti-ADAM9-Antibody MAB-A
GGYYYYFNSGTLDY

SEQ ID NO: 38 - protein, 14 aa, Artificial Sequence
  Alternative CDRH3 Domain of Anti-ADAM9-Antibody MAB-A
GGYYYYIGKGVLDY

SEQ ID NO: 39 - protein, 14 aa, Artificial Sequence
  Alternative CDRH3 Domain of Anti-ADAM9-Antibody MAB-A
GGYYYYPRFGWLDY

SEQ ID NO: 40 - protein, 14 aa, Artificial Sequence
  Alternative CDRH3 Domain of Anti-ADAM9-Antibody MAB-A
GGYYYYTGKGVLDY

SEQ ID NO: 41 - protein, 14 aa, Artificial Sequence
  Alternative CDRH3 Domain of Anti-ADAM9-Antibody MAB-A
GGYYYYDSNAVLDY

SEQ ID NO: 42 - protein, 14 aa, Artificial Sequence
  Alternative CDRH3 Domain of Anti-ADAM9-Antibody MAB-A
GGYYYYFHSGTLDY

SEQ ID NO: 43 - protein, 14 aa, Artificial Sequence
  Alternative CDRH3 Domain of Anti-ADAM9-Antibody MAB-A
GGYYYYFNKAVLDY

SEQ ID NO: 44 - protein, 14 aa, Artificial Sequence
  Alternative CDRH3 Domain of Anti-ADAM9-Antibody MAB-A
GGYYYYGGSGVLDY

SEQ ID NO: 45 - protein, 14 aa, Artificial Sequence
  Alternative CDRH3 Domain of Anti-ADAM9-Antibody MAB-A
GGYYYYPRQGFLDY

SEQ ID NO: 46 - protein, 14 aa, Artificial Sequence
  Alternative CDRH3 Domain of Anti-ADAM9-Antibody MAB-A
GGYYYYYNSGTLDY

SEQ ID NO: 47 - protein, 5 aa, Artificial Sequence
  Consensus CDRH1 Domain of Anti-ADAM9 Antibody MAB-A
  MISC_FEATURE (4)..(4): Xaa is Methionine (M) or Serine (S)
SYWXH

SEQ ID NO: 48 - protein, 17 aa, Artificial Sequence
  Consensus CDRH2 Domain of Anti-ADAM9-Antibody MAB-A
  MISC_FEATURE (6)..(6): Xaa is Asparagine (N) or Phenylalanine (F)
  MISC_FEATURE (14)..(14): Xaa is Lysine (K) or Arginine (R)
  MISC_FEATURE (16)..(16): Xaa is Lysine (K) or Gluatamine (Q)
  MISC_FEATURE (17)..(17): Xaa is Serine (S) or Glycine (G)
EIIPIXGHTNYNEXFXX

SEQ ID NO: 49 - protein, 14 aa, Artificial Sequence
  Consensus CDRH3 Domain of Anti-ADAM9-Antibody MAB-A
  MISC_FEATURE (7)..(7): Xaa is Proline (P), Phenylalanine (F), Tyrosine (Y), Tryptophan (W), Isoleucine (I), Leucine (L), Valine (V), Threonine (T), Glycine (G) or Asparatate (D)
  MISC_FEATURE (8)..(8): Xaa is Lysine (K), Arginine (R), Glycine (G), Asparagine (N), Histidine (H), or Serine (S)
  MISC_FEATURE (9)..(9): Xaa is Phenylalanine (F), Methionine (M), Serine (S), Lysine (K) or Asparagine (N)
  MISC_FEATURE (10)..(10): Xaa is Glycine (G) or Alanine (A)
  MISC_FEATURE (11)..(11): Xaa is Valine (V), Threonine (T), Tryptophan (W) or Phenylalanine (F)
  MISC_FEATURE (12)..(12): Xaa is Methionine (M), Leucine (L) or Lysine (K)
GGYYYYXXXXXXDY

SEQ ID NO: 50 - protein, 453 aa, Artificial Sequence
  Exemplary Humanized/Optimized IgG1 Heavy Chain of a Derivative/Variant of MAB-A Containing the hMAB-A VH (2) Domain
  MISC_FEATURE (453)..(453): Xaa is Lysine (K) or is Absent
EVQLVESGGGLVKPGGSLRLSCAASGFTFSSYWMHWVRQAPGKGLEWVGEIIPIFGHTNYNEKFKSRFTISLDNSKNTLYLQMGSLRAEDTAVYYCARGGYYYYGSRDYFDYWGQGTTVTVSSASTKGPSVFPLAPSSKSTSGGTAALGCLVKDYFPEPVTVSWNSGALTSGVHTFPAVLQSSGLYSLSSVVTVPSSSLGTQTYICNVNHKPSNTKVDKRVEPKSCDKTHTCPPCPAPELLGGPSVFLFPPKPKDTLMISRTPEVTCVVVDVSHEDPEVKFNWYVDGVEVHNAKTKPREEQYNSTYRVVSVLTVLHQDWLNGKEYKCKVSNKALPAPIEKTISKAKGQPREPQVYTLPPSREEMTKNQVSLTCLVKGFYPSDIAVEWESNGQPENNYKTTPPVLDSDGSFFLYSKLTVDKSRWQQGNVFSCSVMHEALHNHYTQKSLSLSPGX

SEQ ID NO: 51 - protein, 453 aa, Artificial Sequence
  Exemplary Humanized/Optimized IgG1 Heavy Chain of a Derivative/Variant of MAB-A Containing the hMAB-A VH (2C) Domain
  MISC_FEATURE (453)..(453): Xaa is Lysine (K) or is Absent
EVQLVESGGGLVKPGGSLRLSCAASGFTFSSYWMHWVRQAPGKGLEWVGEIIPIFGHTNYNEKFKSRFTISLDNSKNTLYLQMGSLRAEDTAVYYCARGGYYYYPRFGWLDYWGQGTTVTVSSASTKGPSVFPLAPSSKSTSGGTAALGCLVKDYFPEPVTVSWNSGALTSGVHTFPAVLQSSGLYSLSSVVTVPSSSLGTQTYICNVNHKPSNTKVDKRVEPKSCDKTHTCPPCPAPELLGGPSVFLFPPKPKDTLMISRTPEVTCVVVDVSHEDPEVKFNWYVDGVEVHNAKTKPREEQYNSTYRVVSVLTVLHQDWLNGKEYKCKVSNKALPAPIEKTISKAKGQPREPQVYTLPPSREEMTKNQVSLTCLVKGFYPSDIAVEWESNGQPENNYKTTPPVLDSDGSFFLYSKLTVDKSRWQQGNVFSCSVMHEALHNHYTQKSLSLSPGX

SEQ ID NO: 52 - protein, 453 aa, Artificial Sequence
  Exemplary Humanized/Optimized IgG1 Heavy Chain of a Derivative/Variant of MAB-A Containing the hMAB-A VH (2I) Domain
  MISC_FEATURE (453)..(453): Xaa is Lysine (K) or is Absent
EVQLVESGGGLVKPGGSLRLSCAASGFTFSSYWMHWVRQAPGKGLEWVGEIIPIFGHTNYNEKFKSRFTISLDNSKNTLYLQMGSLRAEDTAVYYCARGGYYYYPRQGFLDYWGQGTTVTVSSASTKGPSVFPLAPSSKSTSGGTAALGCLVKDYFPEPVTVSWNSGALTSGVHTFPAVLQSSGLYSLSSVVTVPSSSLGTQTYICNVNHKPSNTKVDKRVEPKSCDKTHTCPPCPAPELLGGPSVFLFPPKPKDTLMISRTPEVTCVVVDVSHEDPEVKFNWYVDGVEVHNAKTKPREEQYNSTYRVVSVLTVLHQDWLNGKEYKCKVSNKALPAPIEKTISKAKGQPREPQVYTLPPSREEMTKNQVSLTCLVKGFYPSDIAVEWESNGQPENNYKTTPPVLDSDGSFFLYSKLTVDKSRWQQGNVFSCSVMHEALHNHYTQKSLSLSPGX

SEQ ID NO: 53 - protein, 111 aa, Artificial Sequence
  Humanized/Optimized VL Domain of Murine Anti-ADAM9 Antibody MAB-A
  MISC_FEATURE (24)..(24): Xaa is Lysine (K) or Arginine (R)
  MISC_FEATURE (32)..(32): Xaa is Aspartate (D) or Serine (S))
  MISC_FEATURE (37)..(37): Xaa is Methionine (M) or Leucine (L)
  MISC_FEATURE (96)..(96): Xaa is Histidine (H) or Tyrosine (Y)
  MISC_FEATURE (97)..(97): Xaa is Glutamate (E) or Serine (S)
  MISC_FEATURE (98)..(98): Xaa is Aspattate (D) or Threonine (T)
DIVMTQSPDSLAVSLGERATISCXASQSVDYXGDSYXNWYQQKPGQPPKLLIYAASDLESGIPARFSGSGSGTDFTLTISSLEPEDFATYYCQQSXXXPFTFGQGTKLEIK

SEQ ID NO: 54 - protein, 111 aa, Artificial Sequence
  VL(1) Domain of Humanized/Optimized Anti-ADAM9 Antibody hMAB-A (hMAB-A VL(1))
DIVMTQSPDSLAVSLGERATISCKASQSVDYDGDSYMNWYQQKPGQPPKLLIYAASDLESGIPARFSGSGSGTDFTLTISSLEPEDFATYYCQQSHEDPFTFGQGTKLEIK

SEQ ID NO: 55 - protein, 111 aa, Artificial Sequence
  VL(2) Domain of Humanized/Optimized Anti-ADAM9 Antibody hMAB-A (hMAB-A VL(2))
DIVMTQSPDSLAVSLGERATISCKASQSVDYSGDSYMNWYQQKPGQPPKLLIYAASDLESGIPARFSGSGSGTDFTLTISSLEPEDFATYYCQQSHEDPFTFGQGTKLEIK

SEQ ID NO: 56 - protein, 111 aa, Artificial Sequence
  VL(3) Domain of Humanized/Optimized Anti-ADAM9 Antibody hMAB-A (hMAB-A VL(3))
DIVMTQSPDSLAVSLGERATISCRASQSVDYSGDSYMNWYQQKPGQPPKLLIYAASDLESGIPARFSGSGSGTDFTLTISSLEPEDFATYYCQQSHEDPFTFGQGTKLEIK

SEQ ID NO: 57 - protein, 111 aa, Artificial Sequence
  VL(4) Domain of Humanized/Optimized Anti-ADAM9 Antibody hMAB-A (hMAB-A VL(4))
DIVMTQSPDSLAVSLGERATISCRASQSVDYSGDSYLNWYQQKPGQPPKLLIYAASDLESGIPARFSGSGSGTDFTLTISSLEPEDFATYYCQQSYSTPFTFGQGTKLEIK

SEQ ID NO: 58 - protein, 23 aa, Artificial Sequence
  FRL1 Domain of Humanized/Optimized Murine Anti-ADAM9 Antibody MAB-A
DIVMTQSPDSLAVSLGERATISC

SEQ ID NO: 59 - protein, 15 aa, Artificial Sequence
  FRL2 Domain of Humanized/Optimized Murine Anti-ADAM9 Antibody MAB-A
WYQQKPGQPPKLLIY

SEQ ID NO: 60 - protein, 32 aa, Artificial Sequence
  FRL3 Domain of Humanized/Optimized Murine Anti-ADAM9 Antibody MAB-A
GIPARFSGSGSGTDFTLTISSLEPEDFATYYC

SEQ ID NO: 61 - protein, 10 aa, Artificial Sequence
  FRL4 Domain of Humanized/Optimized Murine Anti-ADAM9 Antibody MAB-A
FGQGTKLEIK

SEQ ID NO: 62 - protein, 15 aa, Artificial Sequence
  Alternative CDRL1 Domain of Anti-ADAM9 Antibody MAB-A
KASQSVDYSGDSYMN

SEQ ID NO: 63 - protein, 15 aa, Artificial Sequence
  Alternative CDRL1 Domain of Anti-ADAM9 Antibody MAB-A
RASQSVDYSGDSYMN

SEQ ID NO: 64 - protein, 15 aa, Artificial Sequence
  Alternative CDRL1 Domain of Anti-ADAM9 Antibody MAB-A
RASQSVDYSGDSYLN

SEQ ID NO: 65 - protein, 9 aa, Artificial Sequence
  Alternative CDRL2 Domain of Anti-ADAM9 Antibody MAB-A
QQSYSTPFT

SEQ ID NO: 66 - protein, 15 aa, Artificial Sequence
  Consensus CDRL1 Domain of Anti-ADAM9 Antibody MAB-A
  MISC_FEATURE (1)..(1): Xaa is Lysine (K) or Arginine (R)
  MISC_FEATURE (9)..(9): Xaa is Aspartate (D) or Serine (S)
  MISC_FEATURE (14)..(14): Xaa is Methionine (M) or Leucine (L)
XASQSVDYXGDSYXN

SEQ ID NO: 67 - protein, 9 aa, Artificial Sequence
  Consensus CDRL3 Domain of Anti-ADAM9 Antibody MAB-A
  MISC_FEATURE (4)..(4): Xaa is Histidine (H) or Tyrosine (Y)
  MISC_FEATURE (5)..(5): Xaa is Glutamate (E) or Serine (S)
  MISC_FEATURE (6)..(6): Xaa is Aspartate (D) or Threonine (T)
QQSXXXPFT

SEQ ID NO: 68 - protein, 218 aa, Artificial Sequence
  Exemplary Humanized/Optimized IgG1 Light Chain of a Derivative/Variant of MAB-A Containing the hMAB-A VL (2) Domain
DIVMTQSPDSLAVSLGERATISCKASQSVDYSGDSYMNWYQQKPGQPPKLLIYAASDLESGIPARFSGSGSGTDFTLTISSLEPEDFATYYCQQSHEDPFTFGQGTKLEIKRTVAAPSVFIFPPSDEQLKSGTASVVCLLNNFYPREAKVQWKVDNALQSGNSQESVTEQDSKDSTYSLSSTLTLSKADYEKHKVYACEVTHQGLSSPVTKSFNRGEC

SEQ ID NO: 69 - protein, 8 aa, Artificial Sequence
  Peferred Intervening Spacer Peptide (Linker 1)
GGGSGGGG

SEQ ID NO: 70 - protein, 6 aa, Artificial Sequence
  Preferred Cysteine-Containing Spacer Peptide (Linker 2)
GGCGGG

SEQ ID NO: 71 - protein, 4 aa, Artificial Sequence
  Alternative Spacer Peptide (Linker 2)
GGGS

SEQ ID NO: 72 - protein, 6 aa, Artificial Sequence
  Alternative Spacer Peptide (Linker 2)
LGGGSG

SEQ ID NO: 73 - protein, 11 aa, Artificial Sequence
  Alternative Spacer Peptide (Linker 2)
GGGSGGGSGGG

SEQ ID NO: 74 - protein, 5 aa, Artificial Sequence
  Alternative Spacer Peptide (Linker 2)
ASTKG

SEQ ID NO: 75 - protein, 6 aa, Artificial Sequence
  Alternative Spacer Peptide (Linker 2)
LEPKSS

SEQ ID NO: 76 - protein, 5 aa, Artificial Sequence
  Alternative Spacer Peptide (Linker 2)
APSSS

SEQ ID NO: 77 - protein, 7 aa, Artificial Sequence
  Heterodimer-Promoting Domain
GVEPKSC

SEQ ID NO: 78 - protein, 6 aa, Artificial Sequence
  Heterodimer-Promoting Domain
VEPKSC

SEQ ID NO: 79 - protein, 6 aa, Artificial Sequence
  Heterodimer-Promoting Domain
AEPKSC

SEQ ID NO: 80 - protein, 7 aa, Artificial Sequence
  Heterodimer-Promoting Domain
GFNRGEC

SEQ ID NO: 81 - protein, 6 aa, Artificial Sequence
  Heterodimer-Promoting Domain
FNRGEC

SEQ ID NO: 82 - protein, 28 aa, Artificial Sequence
  E-Coil Heterodimer-Promoting Domain
EVAALEKEVAALEKEVAALEKEVAALEK

SEQ ID NO: 83 - protein, 28 aa, Artificial Sequence
  K-Coil Heterodimer-Promoting Domain
KVAALKEKVAALKEKVAALKEKVAALKE

SEQ ID NO: 84 - protein, 28 aa, Artificial Sequence
  Cysteine-Containing E-Coil Heterodimer-Promoting Domain
EVAACEKEVAALEKEVAALEKEVAALEK

SEQ ID NO: 85 - protein, 28 aa, Artificial Sequence
  Cysteine-Containing K-Coil Heterodimer-Promoting Domain
KVAACKEKVAALKEKVAALKEKVAALKE

SEQ ID NO: 86 - protein, 46 aa, Streptococcus agalactiae
  MISC_FEATURE (1)..(46): Albumin-Binding Domain 3 (ABD3) of Protein G of Streptococcus strain G148
LAEAKVLANRELDKYGVSDYYKNLIDNAKSAEGVKALIDEILAALP

SEQ ID NO: 87 - protein, 46 aa, Artificial Sequence; identical to SEQ ID NO: 86
  Deimmunized Albumin-Binding Domain 3 (ABD3) of Protein G of Streptococcus strain G148

SEQ ID NO: 88 - protein, 46 aa, Artificial Sequence
  Deimmunized Albumin-Binding Domain 3 (ABD3) of Protein G of Streptococcus strain G148
LAEAKVLANRELDKYGVSDYYKNAANNAKTVEGVKALIAEILAALP

SEQ ID NO: 89 - protein, 46 aa, Artificial Sequence
  Deimmunized Albumin-Binding Domain 3 (ABD3) of Protein G of Streptococcus strain G148
LAEAKVLANRELDKYGVSDYYKNLISNAKSVEGVKALIAEILAALP

SEQ ID NO: 90 - protein, 8 aa, Artificial Sequence
  Linker
APSSSPME

SEQ ID NO: 91 - protein, 16 aa, Artificial Sequence
  Linker
VEPKSADKTHTCPPCP

SEQ ID NO: 92 - protein, 15 aa, Artificial Sequence
  Linker
LEPKSADKTHTCPPC

SEQ ID NO: 93 - protein, 10 aa, Artificial Sequence
  Linker
DKTHTCPPCP

SEQ ID NO: 94 - protein, 13 aa, Artificial Sequence
  Linker
GGGDKTHTCPPCP

SEQ ID NO: 95 - protein, 16 aa, Artificial Sequence
  Linker
LEPKSSDKTHTCPPCP

SEQ ID NO: 96 - protein, 15 aa, Homo sapiens
  MISC_FEATURE (1)..(15): IgG1 Hinge Domain
EPKSCDKTHTCPPCP

SEQ ID NO: 97 - protein, 12 aa, Homo sapiens
  MISC_FEATURE (1)..(12): IgG2 Hinge Domain
ERKCCVECPPCP

SEQ ID NO: 98 - protein, 12 aa, Homo sapiens
  MISC_FEATURE (1)..(12): IgG4 Hinge Domain
ESKYGPPCPSCP

SEQ ID NO: 99 - protein, 12 aa, Artificial Sequence
  Variant IgG4 Hinge Domain
ESKYGPPCPPCP

SEQ ID NO: 100 - protein, 15 aa, Artificial Sequence
  Intervening Spacer Peptide
GGGGSGGGGSGGGGS

SEQ ID NO: 101 - protein, 107 aa, Homo sapiens [sequence omitted]

SEQ ID NO: 102 - protein, 104 aa, Homo sapiens
  MISC_FEATURE (1)..(104): Human IgG CL Lambda Domain
QPKAAPSVTLFPPSSEELQANKATLVCLISDFYPGAVTVAWKADSSPVKAGVETTPSKQSNNKYAASSYLSLTPEQWKSHRSYSCQVTHEGSTVEKTVAPTECS

SEQ ID NO: 103 - protein, 98 aa, Homo sapiens
  MISC_FEATURE (1)..(98): Human IgG1 CH1 Domain
ASTKGPSVFPLAPSSKSTSGGTAALGCLVKDYFPEPVTVSWNSGALTSGVHTFPAVLQSSGLYSLSSVVTVPSSSLGTQTYICNVNHKPSNTKVDKRV

SEQ ID NO: 104 - protein, 98 aa, Homo sapiens
  MISC_FEATURE (1)..(98): Human IgG2 CH1 Domain
ASTKGPSVFPLAPCSRSTSESTAALGCLVKDYFPEPVTVSWNSGALTSGVHTFPAVLQSSGLYSLSSVVTVPSSNFGTQTYTCNVDHKPSNTKVDKTV

SEQ ID NO: 105 - protein, 98 aa, Homo sapiens
  MISC_FEATURE (1)..(98): Human IgG4 CH1 Domain
ASTKGPSVFPLAPCSRSTSESTAALGCLVKDYFPEPVTVSWNSGALTSGVHTFPAVLQSSGLYSLSSVVTVPSSSLGTKTYTCNVDHKPSNTKVDKRV

SEQ ID NO: 106 - protein, 217 aa, Artificial Sequence
  Human IgG1 CH2-CH3 Domain Containing L234A and L235A Substitutions
  MISC_FEATURE (217)..(217): Xaa is Lysine (K) or is Absent
APEAAGGPSVFLFPPKPKDTLMISRTPEVTCVVVDVSHEDPEVKFNWYVDGVEVHNAKTKPREEQYNSTYRVVSVLTVLHQDWLNGKEYKCKVSNKALPAPIEKTISKAKGQPREPQVYTLPPSREEMTKNQVSLTCLVKGFYPSDIAVEWESNGQPENNYKTTPPVLDSDGSFFLYSKLTVDKSRWQQGNVFSCSVMHEALHNHYTQKSLSLSPGX

SEQ ID NO: 107 - protein, 217 aa, Artificial Sequence
  IgG1 CH2-CH3 Domain Containing S442C Substitution
  MISC_FEATURE (217)..(217): Xaa is Lysine (K) or is Absent
APELLGGPSVFLFPPKPKDTLMISRTPEVTCVVVDVSHEDPEVKFNWYVDGVEVHNAKTKPREEQYNSTYRVVSVLTVLHQDWLNGKEYKCKVSNKALPAPIEKTISKAKGQPREPQVYTLPPSREEMTKNQVSLTCLVKGFYPSDIAVEWESNGQPENNYKTTPPVLDSDGSFFLYSKLTVDKSRWQQGNVFSCSVMHEALHNHYTQKSLCLSPGX

SEQ ID NO: 108 - protein, 217 aa, Artificial Sequence
  IgG1 CH2-CH3 Domain Containing L234A, L235A and S442C Substitutions
  MISC_FEATURE (217)..(217): Xaa is Lysine (K) or is Absent
APEAAGGPSVFLFPPKPKDTLMISRTPEVTCVVVDVSHEDPEVKFNWYVDGVEVHNAKTKPREEQYNSTYRVVSVLTVLHQDWLNGKEYKCKVSNKALPAPIEKTISKAKGQPREPQVYTLPPSREEMTKNQVSLTCLVKGFYPSDIAVEWESNGQPENNYKTTPPVLDSDGSFFLYSKLTVDKSRWQQGNVFSCSVMHEALHNHYTQKSLCLSPGX

SEQ ID NO: 109 - protein, 217 aa, Artificial Sequence
  "Knob-Bearing" Variant Human IgG1 CH2-CH3 Domain Containing L234A and L235A Substitutions
  MISC_FEATURE (217)..(217): Xaa is Lysine (K) or is Absent
APEAAGGPSVFLFPPKPKDTLMISRTPEVTCVVVDVSHEDPEVKFNWYVDGVEVHNAKTKPREEQYNSTYRVVSVLTVLHQDWLNGKEYKCKVSNKALPAPIEKTISKAKGQPREPQVYTLPPSREEMTKNQVSLWCLVKGFYPSDIAVEWESNGQPENNYKTTPPVLDSDGSFFLYSKLTVDKSRWQQGNVFSCSVMHEALHNHYTQKSLSLSPGX

SEQ ID NO: 110 - protein, 217 aa, Artificial Sequence
  "Hole-Bearing" Variant Human IgG1 CH2-CH3 Domain Containing L234A and L235A Substitutions
  MISC_FEATURE (217)..(217): Xaa is Lysine (K) or is Absent
APEAAGGPSVFLFPPKPKDTLMISRTPEVTCVVVDVSHEDPEVKFNWYVDGVEVHNAKTKPREEQYNSTYRVVSVLTVLHQDWLNGKEYKCKVSNKALPAPIEKTISKAKGQPREPQVYTLPPSREEMTKNQVSLSCAVKGFYPSDIAVEWESNGQPENNYKTTPPVLDSDGSFFLVSKLTVDKSRWQQGNVFSCSVMHEALHNRYTQKSLSLSPGX

SEQ ID NO: 111 - protein, 118 aa, Artificial Sequence
  VH Domain of Lo-CD2a Anti-Human CD2 Antibody (ATCC Accession No: 11423)
EVQLQQSGPELQRPGASVKLSCKASGYIFTEYYMYWVKQRPKQGLELVGRIDPEDGSIDYVEKFKKKATLTADTSSNTAYMQLSSLTSEDTATYFCARGKFNYRFAYWGQGTLVTVSS

SEQ ID NO: 112 - protein, 112 aa, Artificial Sequence
  VL Domain of Lo-CD2a Anti-Human CD2 Antibody (ATCC Accession No: 11423)
DVVLTQTPPTLLATIGQSVSISCRSSQSLLHSSGNTYLNWLLQRTGQSPQPLIYLVSKLESGVPNRFSGSGSGTDFTLKISGVEAEDLGVYYCMQFTHYPYTFGAGTKLELK

SEQ ID NO: 113 - protein, 125 aa, Artificial Sequence
  VH(1) Domain of Anti-Human CD3 Antibody CD3 mAb-1 (CD3 mAb-1VH(1))
EVQLVESGGGLVQPGGSLRLSCAASGFTFSTYAMNWVRQAPGKGLEWVGRIRSKYNNYATYYADSVKDRFTISRDDSKNSLYLQMNSLKTEDTAVYYCVRHGNFGNSYVSWFAYWGQGTLVTVSS

SEQ ID NO: 114 - protein, 125 aa, Artificial Sequence
  VH(2) Domain of Anti-Human CD3 Antibody CD3 mAb-1 (CD3 mAb-1VH(2))
EVQLVESGGGLVQPGGSLRLSCAASGFTFNTYAMNWVRQAPGKGLEWVARIRSKYNNYATYYADSVKDRFTISRDDSKNSLYLQMNSLKTEDTAVYYCVRHGNFGNSYVSWFAYWGQGTLVTVSS

SEQ ID NO: 115 - protein, 110 aa, Artificial Sequence
  VL Domain of Anti-Human CD3 Antibody CD3 mAb-1
QAVVTQEPSLTVSPGGTVTLTCRSSTGAVTTSNYANWVQQKPGQAPRGLIGGTNKRAPWTPARFSGSLLGGKAALTITGAQAEDEADYYCALWYSNLWVFGGGTKLTVLG

SEQ ID NO: 116 - protein, 125 aa, Artificial Sequence
  VH Domain of Anti-Human CD3 Antibody CD3 mAb-1(D65G)
EVQLVESGGGLVQPGGSLRLSCAASGFTFSTYAMNWVRQAPGKGLEWVGRIRSKYNNYATYYADSVKGRFTISRDDSKNSLYLQMNSLKTEDTAVYYCVRHGNFGNSYVSWFAYWGQGTLVTVSS

SEQ ID NO: 117 - protein, 125 aa, Artificial Sequence
  VH Domain of Anti-Human CD3 mAb-1 Low
EVQLVESGGGLVQPGGSLRLSCAASGFTFSTYAMNWVRQAPGKGLEWVGRIRSKYNNYATYYADSVKGRFTISRDDSKNSLYLQMNSLKTEDTAVYYCVRHGNFGNSYVTWFAYWGQGTLVTVSS

SEQ ID NO: 118 - protein, 125 aa, Artificial Sequence
  VH Domain of Anti-Human CD3 mAb-1 Fast
EVQLVESGGGLVQPGGSLRLSCAASGFTFSTYAMNWVRQAPGKGLEWVGRIRSKYNNYATYYADSVKGRFTISRDDSKNSLYLQMNSLKTEDTAVYYCVRHKNFGNSYVTWFAYWGQGTLVTVSS

SEQ ID NO: 119 - protein, 119 aa, Artificial Sequence [sequence omitted]

SEQ ID NO: 120 - protein, 107 aa, Artificial Sequence
  VL Domain of Anti-Human CD3 mAb-1 OKT3
QIVLTQSPAIMSASPGEKVTMTCSASSSVSYMNWYQQKSGTSPKRWIYDTSKLASGVPAHFRGSGSGTSYSLTISGMEAEDAATYYCQQWSSNPFTFGSGTKLEINR

SEQ ID NO: 121 - protein, 120 aa, Artificial Sequence
  VH Domain of Anti-Human CD8 mAb-1 OKT8
QVQLLESGPELLKPGASVKMSCKASGYTFTDYNMHWVKQSHGKSLEWIGYIYPYTGGTGYNQKFKNKATLTVDSSSSTAYMELRSLTSEDSAVYYCARNFRYTYWYFDVWGQGTTVTVSS

SEQ ID NO: 122 - protein, 112 aa, Artificial Sequence
  VL Domain of Anti-Human CD8 mAb-1 OKT8
DIVMTQSPASLAVSLGQRATISCRASESVDSYDNSLMHWYQQKPGQPPKVLIYLASNLESGVPARFSGSGSRTDFTLTIDPVEADDAATYYCQQNNEDPYTFGGGTKLEIKR

SEQ ID NO: 123 - protein, 121 aa, Artificial Sequence
  VH Domain of Anti-Human CD8 mAb-1 TRX2
QVQLVESGGGVVQPGRSLRLSCAASGFTFSDFGMNWVRQAPGKGLEWVALIYYDGSNKFYADSVKGRFTISRDNSKNTLYLQMNSLRAEDTAVYYCAKPHYDGYYHFFDSWGQGTLVTVSS

SEQ ID NO: 124 - protein, 106 aa, Artificial Sequence
  VL Domain of Anti-Human CD8 mAb-1 TRX2
DIQMTQSPSSLSASVGDRVTITCKGSQDINNYLAWYQQKPGKAPKLLIYNTDILHTGVPSRFSGSGSGTDFTFTISSLQPEDIATYYCYQYNNGYTFGQGTKVEIK

SEQ ID NO: 125 - protein, 118 aa, Artificial Sequence
  VH Domain of Anti-Human CD16 Antibody 3G8
QVTLKESGPGILQPSQTLSLTCSFSGFSLRTSGMGVGWIRQPSGKGLEWLAHIWWDDDKRYNPALKSRLTISKDTSSNQVFLKIASVDTADTATYYCAQINPAWFAYWGQGTLVTVSA

SEQ ID NO: 126 - protein, 111 aa, Artificial Sequence
  VL Domain of Anti-Human CD16 Antibody 3G8
DTVLTQSPASLAVSLGQRATISCKASQSVDFDGDSFMNWYQQKPGQPPKLLIYTTSNLESGIPARFSASGSGTDFTLNIHPVEEEDTATYYCQQSNEDPYTFGGGTKLEIK

SEQ ID NO: 127 - protein, 117 aa, Artificial Sequence
  VH Domain of Anti-Human CD16 Antibody A9
QVQLQQSGAELVRPGTSVKISCKASGYTFTNYWLGWVKQRPGHGLEWIGDIYPGGGYTNYNEKFKGKATVTADTSSRTAYVQVRSLTSEDSAVYFCARSASWYFDVWGARTTVTVSS

SEQ ID NO: 128 - protein, 111 aa, Artificial Sequence
  VL Domain of Anti-Human CD16 Antibody A9
DIQAVVTQESALTTSPGETVTLTCRSNTGTVTTSNYANWVQEKPDHLFTGLIGHTNNRAPGVPARFSGSLIGDKAALTITGAQTEDEAIYFCALWYNNHWVFGGGTKLTVL

SEQ ID NO: 129 - protein, 120 aa, Artificial Sequence
  VH Domain of Anti-Human TCR Antibody BMA 031
QVQLVQSGAEVKKPGASVKVSCKASGYKFTSYVMHWVRQAPGQGLEWIGYINPYNDVTKYNEKFKGRVTITADKSTSTAYLQMNSLRSEDTAVHYCARGSYYDYDGFVYWGQGTLVTVSS

SEQ ID NO: 130 - protein, 106 aa, Artificial Sequence
  VL Domain of Anti-Human TCR Antibody BMA 031
EIVLTQSPATLSLSPGERATLSCSATSSVSYMHWYQQKPGKAPKRWIYDTSKLASGVPSRFSGSGSGTEFTLTISSLQPEDFATYYCQQWSSNPLTFGQGTKLEIK

SEQ ID NO: 131 - protein, 118 aa, Artificial Sequence
  VH Domain of Anti-Human NKG2D Antibody KYK-1.0
EVQLVESGGGVVQPGGSLRLSCAASGFTFSSYGMHWVRQAPGKGLEWVAFIRYDGSNKYYADSVKGRFTISRDNSKNTKYLQMNSLRAEDTAVYYCAKDRFGYYLDYWGQGTLVTVSS

SEQ ID NO: 132 - protein, 108 aa, Artificial Sequence
  VL Domain of Anti-Human NKG2D Antibody KYK-1.0
QPVLTQPSSVSVAPGETARIPCGGDDIETKSVHWYQQKPGQAPVLVIYDDDDRPSGIPERFFGSNSGNTATLSISRVEAGDEADYYCQVWDDNNDEWVFGGGTQLTVL

SEQ ID NO: 133 - protein, 121 aa, Artificial Sequence
  VH Domain of Anti-Human NKG2D Antibody KYK-2.0
QVQLVESGGGLVKPGGSLRLSCAASGFTFSSYGMHWVRQAPGKGLEWVAFIRYDGSNKYYADSVKGRFTISRDNSKNTLYLQMNSLRAEDTAVYYCAKDRGLGDGTYFDYWGQGTTVTVSS

SEQ ID NO: 134 - protein, 110 aa, Artificial Sequence
  VL Domain of Anti-Human NKG2D Antibody KYK-2.0
QSALTQPASVSGSPGQSITISCSGSSSNIGNNAVNWYQQLPGKAPKLLIYYDDLLPSGVSDRFSGSKSGTSAFLAISGLQSEDEADYYCAAWDDSLNGPVFGGGTKLTVL

SEQ ID NO: 135 - protein, 278 aa, Artificial Sequence
  First Polypeptide Chain of ADAM9 x CD3 Bispecific Two-Chain Diabody ("DART-1")
DIVMTQSPDSLAVSLGERATISCKASQSVDYSGDSYMNWYQQKPGQPPKLLIYAASDLESGIPARFSGSGSGTDFTLTISSLEPEDFATYYCQQSHEDPFTFGQGTKLEIKGGGSGGGGEVQLVESGGGLVQPGGSLRLSCAASGFTFSTYAMNWVRQAPGKGLEWVGRIRSKYNNYATYYADSVKGRFTISRDDSKNSLYLQMNSLKTEDTAVYYCVRHGNFGNSYVSWFAYWGQGTLVTVSSGGCGGGEVAALEKEVAALEKEVAALEKEVAALEK

SEQ ID NO: 136 - protein, 275 aa, Artificial Sequence
  Second Polypeptide Chain of ADAM9 x CD3 Bispecific Two-Chain Diabody ("DART-1")
QAVVTQEPSLTVSPGGTVTLTCRSSTGAVTTSNYANWVQQKPGQAPRGLIGGTNKRAPWTPARFSGSLLGGKAALTITGAQAEDEADYYCALWYSNLWVFGGGTKLTVLGGGGSGGGGEVQLVESGGGLVKPGGSLRLSCAASGFTFSSYWMHWVRQAPGKGLEWVGEIIPIFGHTNYNEKFKSRFTISLDNSKNTLYLQMGSLRAEDTAVYYCARGGYYYYGSRDYFDYWGQGTTVTVSSGGCGGGKVAALKEKVAALKEKVAALKEKVAALKE

SEQ ID NO: 137 - protein, 507 aa, Artificial Sequence
  First Polypeptide Chain of ADAM9 x CD3 Bispecific Three-Chain Diabody ("DART-2")
  MISC_FEATURE (507)..(507): Xaa is Lysine (K) or is Absent
DIVMTQSPDSLAVSLGERATISCKASQSVDYSGDSYMNWYQQKPGQPPKLLIYAASDLESGIPARFSGSGSGTDFTLTISSLEPEDFATYYCQQSHEDPFTFGQGTKLEIKGGGSGGGGEVQLVESGGGLVQPGGSLRLSCAASGFTFSTYAMNWVRQAPGKGLEWVGRIRSKYNNYATYYADSVKGRFTISRDDSKNSLYLQMNSLKTEDTAVYYCVRHGNFGNSYVSWFAYWGQGTLVTVSSASTKGEVAACEKEVAALEKEVAALEKEVAALEKGGGDKTHTCPPCPAPEAAGGPSVFLFPPKPKDTLMISRTPEVTCVVVDVSHEDPEVKFNWYVDGVEVHNAKTKPREEQYNSTYRVVSVLTVLHQDWLNGKEYKCKVSNKALPAPIEKTISKAKGQPREPQVYTLPPSREEMTKNQVSLWCLVKGFYPSDIAVEWESNGQPENNYKTTPPVLDSDGSFFLYSKLTVDKSRWQQGNVFSCSVMHEALHNHYTQKSLSLSPGX

SEQ ID NO: 138 - protein, 274 aa, Artificial Sequence
  Second Polypeptide Chain of ADAM9 x CD3 Bispecific Three-Chain Diabody ("DART-2")
QAVVTQEPSLTVSPGGTVTLTCRSSTGAVTTSNYANWVQQKPGQAPRGLIGGTNKRAPWTPARFSGSLLGGKAALTITGAQAEDEADYYCALWYSNLWVFGGGTKLTVLGGGGSGGGGEVQLVESGGGLVKPGGSLRLSCAASGFTFSSYWMHWVRQAPGKGLEWVGEIIPIFGHTNYNEKFKSRFTISLDNSKNTLYLQMGSLRAEDTAVYYCARGGYYYYGSRDYFDYWGQGTTVTVSSASTKGKVAACKEKVAALKEKVAALKEKVAALKE

SEQ ID NO: 139 - protein, 227 aa, Artificial Sequence
  Third Polypeptide Chain of ADAM9 x CD3 Bispecific Three-Chain Diabody ("DART-2")
  MISC_FEATURE (227)..(227): Xaa is Lysine (K) or is Absent
DKTHTCPPCPAPEAAGGPSVFLFPPKPKDTLMISRTPEVTCVVVDVSHEDPEVKFNWYVDGVEVHNAKTKPREEQYNSTYRVVSVLTVLHQDWLNGKEYKCKVSNKALPAPIEKTISKAKGQPREPQVYTLPPSREEMTKNQVSLSCAVKGFYPSDIAVEWESNGQPENNYKTTPPVLDSDGSFFLVSKLTVDKSRWQQGNVFSCSVMHEALHNRYTQKSLSLSPGX

SEQ ID NO: 140 - protein, 6 aa, Artificial Sequence
  Sub-Domain Portion of CDRH3 Domain of anti-Human ADAM9 Antibody MAB-A (2.2)
GSRDYF

SEQ ID NO: 141 - protein, 6 aa, Artificial Sequence
  Variant of Sub-Domain Portion of CDRH3 Domain of Anti-Human ADAM9 Antibody hMAB-A (2.2)
DGEGVM

SEQ ID NO: 142 - protein, 6 aa, Artificial Sequence
  Variant of Sub-Domain Portion of CDRH3 Domain of Anti-Human ADAM9 Antibody hMAB-A (2.2)
FHSGLL

SEQ ID NO: 143 - protein, 6 aa, Artificial Sequence
  Variant of Sub-Domain Portion of CDRH3 Domain of Anti-Human ADAM9 Antibody hMAB-A (2.2)
FNSATL

SEQ ID NO: 144 - protein, 6 aa, Artificial Sequence
  Variant of Sub-Domain Portion of CDRH3 Domain of Anti-Human ADAM9 Antibody hMAB-A (2.2)
FNSGTL

SEQ ID NO: 145 - protein, 6 aa, Artificial Sequence
  Variant of Sub-Domain Portion of CDRH3 Domain of Anti-Human ADAM9 Antibody hMAB-A (2.2)
FNSSTL

SEQ ID NO: 146 - protein, 6 aa, Artificial Sequence
  Variant of Sub-Domain Portion of CDRH3 Domain of Anti-Human ADAM9 Antibody hMAB-A (2.2)
GKSKWL

SEQ ID NO: 147 - protein, 6 aa, Artificial Sequence
  Variant of Sub-Domain Portion of CDRH3 Domain of Anti-Human ADAM9 Antibody hMAB-A (2.2)
GMGGTL

SEQ ID NO: 148 - protein, 6 aa, Artificial Sequence
  Variant of Sub-Domain Portion of CDRH3 Domain of Anti-Human ADAM9 Antibody hMAB-A (2.2)
HAKGGM

SEQ ID NO: 149 - protein, 6 aa, Artificial Sequence
  Variant of Sub-Domain Portion of CDRH3 Domain of Anti-Human ADAM9 Antibody hMAB-A (2.2)
IGEAVL

SEQ ID NO: 150 - protein, 6 aa, Artificial Sequence
  Variant of Sub-Domain Portion of CDRH3 Domain of Anti-Human ADAM9 Antibody hMAB-A (2.2)
IGKGVF

SEQ ID NO: 151 - protein, 6 aa, Artificial Sequence
  Variant of Sub-Domain Portion of CDRH3 Domain of Anti-Human ADAM9 Antibody hMAB-A (2.2)
IGKGVL

SEQ ID NO: 152 - protein, 6 aa, Artificial Sequence
  Variant of Sub-Domain Portion of CDRH3 Domain of Anti-Human ADAM9 Antibody hMAB-A (2.2)
KHDSVL

SEQ ID NO: 153 - protein, 6 aa, Artificial Sequence
  Variant of Sub-Domain Portion of CDRH3 Domain of Anti-Human ADAM9 Antibody hMAB-A (2.2)
LNTAVM

SEQ ID NO: 154 - protein, 6 aa, Artificial Sequence
  Variant of Sub-Domain Portion of CDRH3 Domain of Anti-Human ADAM9 Antibody hMAB-A (2.2)
NGEGTL

SEQ ID NO: 155 - protein, 6 aa, Artificial Sequence
  Variant of Sub-Domain Portion of CDRH3 Domain of Anti-Human ADAM9 Antibody hMAB-A (2.2)
NGKNTL

SEQ ID NO: 156 - protein, 6 aa, Artificial Sequence
  Variant of Sub-Domain Portion of CDRH3 Domain of Anti-Human ADAM9 Antibody hMAB-A (2.2)
NSAGIL

SEQ ID NO: 157 - protein, 6 aa, Artificial Sequence
  Variant of Sub-Domain Portion of CDRH3 Domain of Anti-Human ADAM9 Antibody hMAB-A (2.2)
PKEGWM

SEQ ID NO: 158 - protein, 6 aa, Artificial Sequence
  Variant of Sub-Domain Portion of CDRH3 Domain of Anti-Human ADAM9 Antibody hMAB-A (2.2)
PKFGWK

SEQ ID NO: 159 - protein, 6 aa, Artificial Sequence
  Variant of Sub-Domain Portion of CDRH3 Domain of Anti-Human ADAM9 Antibody hMAB-A (2.2)
PKMGWV

SEQ ID NO: 160 - protein, 6 aa, Artificial Sequence
  Variant of Sub-Domain Portion of CDRH3 Domain of Anti-Human ADAM9 Antibody hMAB-A (2.2)
PRLGHL

SEQ ID NO: 161 - protein, 6 aa, Artificial Sequence
  Variant of Sub-Domain Portion of CDRH3 Domain of Anti-Human ADAM9 Antibody hMAB-A (2.2)
PSFGWA

SEQ ID NO: 162 - protein, 6 aa, Artificial Sequence
  Variant of Sub-Domain Portion of CDRH3 Domain of Anti-Human ADAM9 Antibody hMAB-A (2.2)
QAKGTM

SEQ ID NO: 163 - protein, 6 aa, Artificial Sequence
  Variant of Sub-Domain Portion of CDRH3 Domain of Anti-Human ADAM9 Antibody hMAB-A (2.2)
RGMGVM

SEQ ID NO: 164 - protein, 6 aa, Artificial Sequence
  Variant of Sub-Domain Portion of CDRH3 Domain of Anti-Human ADAM9 Antibody hMAB-A (2.2)
RKEGWM

SEQ ID NO: 165 - protein, 6 aa, Artificial Sequence
  Variant of Sub-Domain Portion of CDRH3 Domain of Anti-Human ADAM9 Antibody hMAB-A (2.2)
TGKGVL

SEQ ID NO: 166 - protein, 6 aa, Artificial Sequence
  Variant of Sub-Domain Portion of CDRH3 Domain of Anti-Human ADAM9 Antibody hMAB-A (2.2)
TGMGTL

SEQ ID NO: 167 - protein, 6 aa, Artificial Sequence
  Variant of Sub-Domain Portion of CDRH3 Domain of Anti-Human ADAM9 Antibody hMAB-A (2.2)
TGNGVM

SEQ ID NO: 168 - protein, 6 aa, Artificial Sequence
  Variant of Sub-Domain Portion of CDRH3 Domain of Anti-Human ADAM9 Antibody hMAB-A (2.2)
WNAGTF

SEQ ID NO: 169 - protein, 6 aa, Artificial Sequence
  Variant of Sub-Domain Portion of CDRH3 Domain of Anti-Human ADAM9 Antibody hMAB-A (2.2)
YHHTPL

SEQ ID NO: 170 - protein, 6 aa, Artificial Sequence
  Variant of Sub-Domain Portion of CDRH3 Domain of Anti-Human ADAM9 Antibody hMAB-A (2.2)
YQSATL

SEQ ID NO: 171 - protein, 6 aa, Artificial Sequence
  Variant of Sub-Domain Portion of CDRH3 Domain of Anti-Human ADAM9 Antibody hMAB-A (2.2)
DGKAVL

SEQ ID NO: 172 - protein, 6 aa, Artificial Sequence
  Variant of Sub-Domain Portion of CDRH3 Domain of Anti-Human ADAM9 Antibody hMAB-A (2.2)
FNKAVL

SEQ ID NO: 173 - protein, 6 aa, Artificial Sequence
  Variant of Sub-Domain Portion of CDRH3 Domain of Anti-Human ADAM9 Antibody hMAB-A (2.2)
FNSGTW

SEQ ID NO: 174 - protein, 6 aa, Artificial Sequence
  Variant of Sub-Domain Portion of CDRH3 Domain of Anti-Human ADAM9 Antibody hMAB-A (2.2)
FNTGVF

SEQ ID NO: 175 - protein, 6 aa, Artificial Sequence
  Variant of Sub-Domain Portion of CDRH3 Domain of Anti-Human ADAM9 Antibody hMAB-A (2.2)
GKSRFH

SEQ ID NO: 176 - protein, 6 aa, Artificial Sequence
  Variant of Sub-Domain Portion of CDRH3 Domain of Anti-Human ADAM9 Antibody hMAB-A (2.2)
IGKNVY

SEQ ID NO: 177 - protein, 6 aa, Artificial Sequence
  Variant of Sub-Domain Portion of CDRH3 Domain of Anti-Human ADAM9 Antibody hMAB-A (2.2)
MGKGVM

SEQ ID NO: 178 - protein, 6 aa, Artificial Sequence
  Variant of Sub-Domain Portion of CDRH3 Domain of Anti-Human ADAM9 Antibody hMAB-A (2.2)
NGESVF

SEQ ID NO: 179 - protein, 6 aa, Artificial Sequence
  Variant of Sub-Domain Portion of CDRH3 Domain of Anti-Human ADAM9 Antibody hMAB-A (2.2)
PDFGWM

SEQ ID NO: 180 - protein, 6 aa, Artificial Sequence
  Variant of Sub-Domain Portion of CDRH3 Domain of Anti-Human ADAM9 Antibody hMAB-A (2.2)
PGSGVM

SEQ ID NO: 181 - protein, 6 aa, Artificial Sequence
  Variant of Sub-Domain Portion of CDRH3 Domain of Anti-Human ADAM9 Antibody hMAB-A (2.2)
PKDAWL

SEQ ID NO: 182 - protein, 6 aa, Artificial Sequence
  Variant of Sub-Domain Portion of CDRH3 Domain of anti-Human ADAM9 Antibody MAB-A
PKFGWL

SEQ ID NO: 183 - protein, 6 aa, Artificial Sequence
  Variant of Sub-Domain Portion of CDRH3 Domain of anti-Human ADAM9 Antibody MAB-A
PKIGWH

SEQ ID NO: 184 - protein, 6 aa, Artificial Sequence
  Variant of Sub-Domain Portion of CDRH3 Domain of Anti-Human ADAM9 Antibody hMAB-A (2.2)
PKMGWA

SEQ ID NO: 185 - protein, 6 aa, Artificial Sequence
  Variant of Sub-Domain Portion of CDRH3 Domain of Anti-Human ADAM9 Antibody hMAB-A (2.2)
PKMGWM

SEQ ID NO: 186 - protein, 6 aa, Artificial Sequence
  Variant of Sub-Domain Portion of CDRH3 Domain of Anti-Human ADAM9 Antibody hMAB-A (2.2)
PQMGWL

SEQ ID NO: 187 - protein, 6 aa, Artificial Sequence
  Variant of Sub-Domain Portion of CDRH3 Domain of Anti-Human ADAM9 Antibody hMAB-A (2.2)
PRFGWL

SEQ ID NO: 188 - protein, 6 aa, Artificial Sequence
  Variant of Sub-Domain Portion of CDRH3 Domain of Anti-Human ADAM9 Antibody hMAB-A (2.2)
PRMGFL

SEQ ID NO: 189 - protein, 6 aa, Artificial Sequence
  Variant of Sub-Domain Portion of CDRH3 Domain of Anti-Human ADAM9 Antibody hMAB-A (2.2)
PRMGFM

SEQ ID NO: 190 - protein, 6 aa, Artificial Sequence
  Variant of Sub-Domain Portion of CDRH3 Domain of Anti-Human ADAM9 Antibody hMAB-A (2.2)
PSFGWM

SEQ ID NO: 191 - protein, 6 aa, Artificial Sequence
  Variant of Sub-Domain Portion of CDRH3 Domain of Anti-Human ADAM9 Antibody hMAB-A (2.2)
RREGWM

SEQ ID NO: 192 - protein, 6 aa, Artificial Sequence
  Variant of Sub-Domain Portion of CDRH3 Domain of Anti-Human ADAM9 Antibody hMAB-A (2.2)
SGEGVL

SEQ ID NO: 193 - protein, 6 aa, Artificial Sequence
  Variant of Sub-Domain Portion of CDRH3 Domain of Anti-Human ADAM9 Antibody hMAB-A (2.2)
SGNGVM

SEQ ID NO: 194 - protein, 6 aa, Artificial Sequence
  Variant of Sub-Domain Portion of CDRH3 Domain of Anti-Human ADAM9 Antibody hMAB-A (2.2)
VGKAVL

SEQ ID NO: 195 - protein, 6 aa, Artificial Sequence
  Variant of Sub-Domain Portion of CDRH3 Domain of Anti-Human ADAM9 Antibody hMAB-A VH (2E)
DSNAVL

SEQ ID NO: 196 - protein, 6 aa, Artificial Sequence
  Variant of Sub-Domain Portion of CDRH3 Domain of Anti-Human ADAM9 Antibody hMAB-A VH (2F)
FHSGTL

SEQ ID NO: 197 - protein, 6 aa, Artificial Sequence
  Variant of Sub-Domain Portion of CDRH3 Domain of Anti-Human ADAM9 Antibody hMAB-A VH (2H)
GGSGVL

SEQ ID NO: 198 - protein, 6 aa, Artificial Sequence
  Variant of Sub-Domain Portion of CDRH3 Domain of Anti-Human ADAM9 Antibody hMAB-A VH (2I)
PRQGFL

SEQ ID NO: 199 - protein, 6 aa, Artificial Sequence
  Variant of Sub-Domain Portion of CDRH3 Domain of Anti-Human ADAM9 Antibody hMAB-A VH (2J)
YNSGTL

SEQ ID NO: 200 - protein, 217 aa, Artificial Sequence
  Human IgG1 CH2-CH3 Domain Containing M252Y/S254T/T256E Substitutions
  MISC_FEATURE (217)..(217): Xaa is Lysine (K) or is Absent
APELLGGPSVFLFPPKPKDTLYITREPEVTCVVVDVSHEDPEVKFNWYVDGVEVHNAKTKPREEQYNSTYRVVSVLTVLHQDWLNGKEYKCKVSNKALPAPIEKTISKAKGQPREPQVYTLPPSREEMTKNQVSLTCLVKGFYPSDIAVEWESNGQPENNYKTTPPVLDSDGSFFLYSKLTVDKSRWQQGNVFSCSVMHEALHNHYTQKSLSLSPGX

SEQ ID NO: 201 - protein, 217 aa, Artificial Sequence
  Human IgG1 CH2-CH3 Domain Containing L234A/L235A/M252Y/S254T/T256E Substitutions
  MISC_FEATURE (217)..(217): Xaa is Lysine (K) or is Absent
APEAAGGPSVFLFPPKPKDTLYITREPEVTCVVVDVSHEDPEVKFNWYVDGVEVHNAKTKPREEQYNSTYRVVSVLTVLHQDWLNGKEYKCKVSNKALPAPIEKTISKAKGQPREPQVYTLPPSREEMTKNQVSLTCLVKGFYPSDIAVEWESNGQPENNYKTTPPVLDSDGSFFLYSKLTVDKSRWQQGNVFSCSVMHEALHNHYTQKSLSLSPGX

SEQ ID NO: 202 - protein, 453 aa, Artificial Sequence
  Humanized/Optimized IgG1 Heavy Chain of hMAB-A VH (2I) Containing L234A/L235A Substitutions
  MISC_FEATURE (453)..(453): Xaa is Lysine (K) or is Absent
EVQLVESGGGLVKPGGSLRLSCAASGFTFSSYWMHWVRQAPGKGLEWVGEIIPIFGHTNYNEKFKSRFTISLDNSKNTLYLQMGSLRAEDTAVYYCARGGYYYYPRQGFLDYWGQGTTVTVSSASTKGPSVFPLAPSSKSTSGGTAALGCLVKDYFPEPVTVSWNSGALTSGVHTFPAVLQSSGLYSLSSVVTVPSSSLGTQTYICNVNHKPSNTKVDKRVEPKSCDKTHTCPPCPAPEAAGGPSVFLFPPKPKDTLMISRTPEVTCVVVDVSHEDPEVKFNWYVDGVEVHNAKTKPREEQYNSTYRVVSVLTVLHQDWLNGKEYKCKVSNKALPAPIEKTISKAKGQPREPQVYTLPPSREEMTKNQVSLTCLVKGFYPSDIAVEWESNGQPENNYKTTPPVLDSDGSFFLYSKLTVDKSRWQQGNVFSCSVMHEALHNHYTQKSLSLSPGX

SEQ ID NO: 203 - protein, 217 aa, Artificial Sequence
  Human IgG1 CH2-CH3 Domain Containing L234A, L235A, M252Y, S254T, T256E and S442C Substitutions
  MISC_FEATURE (217)..(217): Xaa is Lysine (K) or is Absent
APEAAGGPSVFLFPPKPKDTLYITREPEVTCVVVDVSHEDPEVKFNWYVDGVEVHNAKTKPREEQYNSTYRVVSVLTVLHQDWLNGKEYKCKVSNKALPAPIEKTISKAKGQPREPQVYTLPPSREEMTKNQVSLTCLVKGFYPSDIAVEWESNGQPENNYKTTPPVLDSDGSFFLYSKLTVDKSRWQQGNVFSCSVMHEALHNHYTQKSLCLSPGX

SEQ ID NO: 204 - protein, 217 aa, Artificial Sequence
  "Knob-Bearing" Variant Human IgG1 CH2-CH3 Domain Containing L234A, L235A, M252Y, S254Tand T256E Substitutions
  MISC_FEATURE (217)..(217): Xaa is Lysine (K) or is Absent
APEAAGGPSVFLFPPKPKDTLYITREPEVTCVVVDVSHEDPEVKFNWYVDGVEVHNAKTKPREEQYNSTYRVVSVLTVLHQDWLNGKEYKCKVSNKALPAPIEKTISKAKGQPREPQVYTLPPSREEMTKNQVSLWCLVKGFYPSDIAVEWESNGQPENNYKTTPPVLDSDGSFFLYSKLTVDKSRWQQGNVFSCSVMHEALHNHYTQKSLSLSPGX

SEQ ID NO: 205 - protein, 217 aa, Artificial Sequence
  "Hole-Bearing" Variant Human IgG1 CH2-CH3 Domain Containing L234A, L235A, M252Y, S254Tand T256E Substitutions
  MISC_FEATURE (217)..(217): Xaa is Lysine (K) or is Absent
APEAAGGPSVFLFPPKPKDTLYITREPEVTCVVVDVSHEDPEVKFNWYVDGVEVHNAKTKPREEQYNSTYRVVSVLTVLHQDWLNGKEYKCKVSNKALPAPIEKTISKAKGQPREPQVYTLPPSREEMTKNQVSLSCAVKGFYPSDIAVEWESNGQPENNYKTTPPVLDSDGSFFLVSKLTVDKSRWQQGNVFSCSVMHEALHNRYTQKSLSLSPGX

SEQ ID NO: 206 - protein, 62 aa, Homo sapiens
  MISC_FEATURE (1)..(52): IgG3 Hinge Domain
ELKTPLGDTTHTCPRCPEPKSCDTPPPCPRCPEPKSCDTPPPCPRCPEPKSCDTPPPCPRCP

SEQ ID NO: 207 - protein, 98 aa, Homo sapiens
  MISC_FEATURE (1)..(98): Human IgG3 Domain
ASTKGPSVFPLAPCSRSTSGGTAALGCLVKDYFPEPVTVSWNSGALTSGVHTFPAVLQSSGLYSLSSVVTVPSSSLGTQTYTCNVNHKPSNTKVDKRV